European Patent Specification EP 3 548 639 B9, published October 4, 2023. Title: BACTERIAL STRAINS AND CONSORTIUM COMPRISING SAME FOR DEGRADING MTBE, TBA AND/OR HCHO. Applicant: VITO NV. The sequence listing filed with the application follows.

SEQUENCE LISTING (3 sequences)

SEQ ID NO: 1 - DNA, 1661 bp, Methylibium sp.
tgaattgtaatacgactcactatagggcgaattgggccctctagatgcatgctcgagcggccgccagtgtgatggatatctgcagaattcgcccttagagtttgatcctggctcagattgaacgctggcggcatgccttacacatgcaagtcgaacggcagcacgggagcaatcctggtggcgagtggcgaacgggtgagtaatacatcggaacgtgcccagttgtgggggatagcccggcgaaagccggattaataccgcatacgacctacgggtgaaagcgggggatcgcaagacctcgcgctattggagcggccgatgtcggattagctagttggtggggtaaaagcctaccaaggctacgatccgtagctggtctgagaggacgaccagccacactgggactgagacacggcccagactcctacgggaggcagcagtggggaattttggacaatgggcgcaagcctgatccagccatgccgcgtgcgggaagaaggccttcgggttgtaaaccgcttttgtcagggaagaaacggtttgggctaataccccgaactaatgacggtacctgaagaataagcaccggctaactacgtgccagcagccgcggtaatacgtagggtgcaagcgttaatcggaattactgggcgtaaagcgtgcgcaggcggctttgcaagacagatgtgaaatccccgggctcaacctgggaactgcatttgtgactgcaaggctggagtgcggcagagggggatggaattccgcgtgtagcagtgaaatgcgtagatatgcggaggaacaccgatggcgaaggcaatcccctgggcctgcactgacgctcatgcacgaaagcgtggggagcaaacaggattagataccctggtagtccacgccctaaacgatgtcaactggttgttggacggcttgctgttcagtaacgaagctaacgcgtgaagttgaccgcctggggagtacggccgcaaggttgaaactcaaaggaattgacggggacccgcacaagcggtggatgatgtggtttaattcgatgcaacgcgaaaaaccttacctacccttgacatgtctagaagttaccagagatggtttcgtgctcgaaagagaactagaacacaggtgctgcatggccgtcgtcagctcgtgtcgtgagatgttgggttaagtcccgcaacgagcgcaacccttgtcattagttgctacgtaagggcactctaatgagactgccggtgacaaaccggaggaaggtggggatgacgtcaggtcatcatggcccttatgggtagggctacacacgtcatacaatggccggtacagagggctgccaacccgcgagggggagccaatcccagaaaaccggtcgtagtccggatcgcagtctgcaactcgactgcgtgaagtcggaatcgctagtaatcgcggatcagcttgccgcggtgaatacgttcctgggtcttgtacacaccgcccgtcacaccatgggagcgggttctgccagaagtagttagcctaaccgcaaggagggcgattaccacggcagggttcgtgactggggtgaagtcgtaacaaggtaaccaagggcgaattccagcacactggcggccgttactagtggatccgagctcggtaccaagcttggcgtaatcatg

SEQ ID NO: 2 - DNA, 1665 bp, Hydrogenophaga sp.
catgattacgccaagcttggtaccgagctcggatccactagtaacggccgccagtgtgctggaattcgcccttagagtttgatcctggctcagattgaacgctggcggcatgctttacacatgcaagtcgaacggtaacaggccgcaaggtgctgacgagtggcgaacgggtgagtaatgcatcggaacgtgcccagtcgtgggggataacgcagcgaaagctgtgctaataccgcatacgatctatggatgaaagcgggggaccgtaaggcctcgcgcgattggagcggccgatgtcagattagctagttggtggggtaaaggcccaccaaggcgacgatctgtagctggtctgagaggacgaccagccacactgggactgagacacggcccagactcctacgggaggcagcagtggggaattttggacaatgggcgcaagcctgatccagcaatgccgcgtgcaggaagaaggccttcgggttgtaaactgcttttgtacggaacgaaacggtctgggttaatacctcgggctaatgacggtaccgtaagaataagcaccggctaactacgtgccagcagccgcggtaatacgtagggtgcaagcgttaatcggaattactgggcgtaaagcgtgcgcaggcggtgatgtaagacagtcgtgaaatccccgggctcaacctgggaattgcgattgtgactgcatcgctggagtgcggcagagggggatggaattccgcgtgtagcagtgaaatgcgtagatatgcggaggaacaccgatggcgaaggcaatcccctgggcctgcactgacgctcatgcacgaaagcgtggggagcaaacaggattagataccctggtagtccacgccctaaacgatgtcaactggttgttgggtctcttctgactcagtaacgaagctaacgcgtgaagttgaccgcctggggagtacggccgcaaggttgaaactcaaaggaattgacggggacccgcacaagcggtggatgatgtggtttaattcgatgcaacgcgaaaaaccttacccacctttgacatgtacggaatttgccagagatggcttagtgctcgaaagagaaccgtaacacaggtgctgcatggctgtcgtcagctcgtgtcgtgagatgttgggttaagtcccgcaacgagcgcaacccttgtcattagttgctacattcagttgggcactctaatgagactgccggtgacaaaccggaggaaggtggggatgacgtcaagtcctcatggcccttataggtggggctacacacgtcatacaatggccggtacaaagggtcgcaaacccgcgagggggagccaatccatcaaagccggtcgtagtccggatcgcagtctgcaactcgactgcgtgaagtcggaatcgctagtaatcgtggatcagcatgtcacggtgaatacgttcccgggtcttgtacacaccgcccgtcacaccatgggagcgggtctcgccagaagtagttagcctaaccgcaaggagggcgattaccacggcggggttcgtgactggggtgaagtcgtaacaaggtagccgtaagggcgaattctgcagatatccatcacactggcggccgctcgagcatgcatctagagggcccaattcgccctatagtgagtcgtattacaattca

SEQ ID NO: 3 - DNA, 1652 bp, Mycobacterium sp.
tgaattgtaatacgactcactatagggcgaattgggccctctagatgcatgctcgagcggccgccagtgtgatggatatctgcagaattcgcccttagagtttgatcctggctcaggacgaacgctggcggcgtgcttaacacatgcaagtcgaacggaaaggcccttcggggtgctcgagtggcgaacgggtgagtaacacgtgggtgatctgccctgcactttgggataagcctgggaaactgggtctaataccgaataggactccggactgcatggtctggggtggaaagcttttgcggtgtgggatgggcccgcggcctatcagcttgttggtggggtgatggcctaccaaggcgacgacgggtagccggcctgagagggtgaccggccacactgggactgagatacggcccagactcctacgggaggcagcagtggggaatattgcacaatgggcgcaagcctgatgcagcgacgccgcgtgagggatgacggccttcgggttgtaaacctctttcagcacagacgaagcgcaagtgacggtatgtgcagaagaaggaccggccaactacgtgccagcagccgcggtaatacgtagggtccgagcgttgtccggaattactgggcgtaaagagctcgtaggtggtttgtcgcgttgttcgtgaaaactcacagcttaactgtgggcgtgcgggcgatacgggcagactggagtactgcaggggagactggaattcctggtgtagcggtggtatgcgcagatatcaggaggaacaccggtggcgaaggcgggtctctgggcagtaactgacgctgaggagcgaaagcgtggggagcgaacaggattagataccctggtagtccacgccgtaaacggtgggtactaggtgtgggtttccttccttgggatccgtgccgtagctaacgcattaagtaccccgcctggggagtacggccgcaaggctaaaactcaaaggaattgacgggggcccgcacaagcggcggagcatgtggattaattcgatgcaacgcgaagaaccttacctgggtttgacatgcacaggacgccggcagagatgtcggttcccttgtggcctgtgtgcaggtggtgcatggctgtcgtcagctcgtgtcgtgagatgttgggttaagtcccgcaacgagcgcaacccttgtctcatgttgccagcacgttatggtggggactcgtgagagactgccggggtcaactcggaggaaggtggggatgacgtcaagtcatcatgccccttatgtccagggcttcacacatgctacaatggccggtacaaagggctgcgatgccgtgaggtggagcgaatcctttcaaagccggtctcagttcggatcggggtctgcaactcgaccccgtgaagtcggagtcgctagtaatcgcagatcagcaacgctgcggtgaatacgttcccgggccttgtacacaccgcccgtcacgtcatgaaagtcggtaacacccgaagccggtggcctaaccccttgtgggagggagccgtcgaaggtgggatcggcgattgggacgaagtcgtaacaaggtagccgtaagggcgaattccagcacactggcggccgttactagtggatccgagctcggtaccaagcttggcgtaatcatg